European Patent Specification EP 3 878 954 B1, published September 2, 2026. Title: ENZYME GENE FOR BIOSYNTHESIS OF CROCIN AND USE THEREOF. Applicant: INSTITUTE OF MEDICINAL PLANT DEVELOPMENT,CHINESE ACADEMY OF MEDICAL SCIENCES. The sequence listing filed with the application follows.

SEQUENCE LISTING (8 sequences)

SEQ ID NO: 1 - DNA, 1995 bp, Gardenia jasminoides
atgactgatttattgtgtttcctatacgaatcgcttggagcacagcataaatactctcctccattatacacattcacccatccatccatccatcttctcttagtgttacaaaacaacaatacaaagacagcaatggatgctttctcttcctctttcctctctcgactatcccaaaatcccaaacttccgacttctctaaccaacccttcatcaccaaatattcctttactacacatttcatccgctagaattgaagataagccacaaccaacaattattactagcacccccatcactgccacaacgccaccatcatctaattctaatccccttaagaagcagaacctaccgaaatatacacttaaaagatccaatcccaagccgcaatcatcatcacaaccaccaccatcactgcagctgcaagaaccttcaagaaagccagtagaaccatcattgctcaccaaattcttcaatgcacttgataacttcatagacacatgcattgatcctccaactcacccttctgttgaccccaaatacgtcctggcaaacaactttgtaccagttgatgaactccccccgaccgaatgtgaggtggtggaaggctttcttccaccgtgccttgacggtgcctacttccgcaatggcccaaaccctcagttcgtcactcacgggccctaccactttttcgatggcgatggaatgatacattccatcaaaatctccgaaggaaaagccaccttctgcagccggtacgtgaaaacatacaagtacatgacggaacgggatacgggctctcccgtgttccctaaagtattctctggtttcaatggcctaacagcctccgcagccagggttgccctagctgctgccagaatgttagctggccaatttaaccgagccaatggttttggcctggcaaacactagcttggctctagttggggggaaactattcgctttaggtgaaccagaccttccatatgctgtaaaattaacacaaactggagatttagtaaccgtaggccgtcatgactttgatggtaagcttattgcgagcatgactgcacatcccaaaatcgaccctgagacaggtgaagctttcgcattcagatacgcgctaatgcctccatttctaaccttctttagaatcaaccctgatggtacaaaagaaccagacgtcccgattttctccatgacacggccttcatttgttcatgatttggccatcacaagaaaatacgctatttttcctgacatacaaatagggatcaaccctcttcagatgatcgccggcggaccactagtgggttcagatccccgaaaagtgccacgactcggggttattcccaggtatgctgcggatgaagctgagatgaagtggtttgatgttccgggacttaatcttatgcatgctgtcaatgcttgggatgaagatgatggtgatggtattgttgttgtaggaactaatagtttgcccattgagcatgttcttcggcggatggatttggttcatgcatccatggtgaaaatcaagattgatctcaagactgggatggtttggaaacatccaatttctacgaggagtatggaatttggagtcattaatccggcttatgttggcaagaagaacaagtatgtatatgcagcagttgtagaccctttgccaaaggtgtcaggagtggtgaagctagacttatcagcttcggcaggtgagcaccgcgactgcgtcattgctagccagctgtatgaaccggagtgctttggaagcgaaccatttttcgtggccaaagaccctaacaacccaaatgcagatgaagatgatggttatgtggtgtcctatgtccatgatgaaaacacaggagagtcaagattcttagtgatggacgcgaagtcaccgagtcttgaaattgtggctgctgtaaaattgcctcaaagggttccttctggctttcatggcctctttgtcagagaaagtgagctcaataaattgtaa

SEQ ID NO: 2 - DNA, 1512 bp, Gardenia jasminoides
atggccgtccaaagcaacggcaatggaagctcggattctcatgttaaggttcctcagataaagttcaccaagctcttcatcaatggagagttcgttgattctgtttcaggaaagacgtttgagacaatagatccaagaaatggggaggtgattgcagaaattgccgaggggggcaaggaagatgttgatttggctgtcaaagctgcccgagaagcttttgaccacggcccatggcctcgtttacctggctctgagaggcgaaagataatgatgaagtttgcagacttaatagatgaaaatacccaagaattggccaccttggatgcaattgatgctggaaaattgttttacctttgcaagattatggatattccaggagcagcagaaacaattcgctattatgcgggtgcggcagataagattcatggggagactctaaaaatgtcaaccgcgctacaaggatacacattgcatgagcccattggagttgttggacacatcattccctggaacttccccagtcaaatgtttgctatgaaggttggccctgcattagcagctggctgcaccatggtagtcaagcctgctgaacagacgcctctgtcagccctctattacgctcatttagcaaagctggctggaatccccgatggagtgctaaacgttgtaacaggattcggacaaacagctggtgcggcaattagctctcatatggacattgatatggtaagtttcacgggttctacagaagtagggcgtctcgtcatgcaagctgcagcaacaagcaacttaaagcctgtgtgtctagaactgggaggcaagtcccccattttaatcttcgatgatgcagatgttgacaaagttacagaactcgcactgcagggaactctatttaacaagggtgaaatatgtgttgctggctctcgtatttttgttcaagaggggatttatgacaagtttttaatcaagttgaagcagaaggtgaagaattgggtggtcggtgacccttttgatccaacatctcatcaaggaccccaagttgacaagaagcagtacgatagaatactttcatacatcgagcatgggaagaaggaaggtgccaccttattccacggtggcaagccttgtgacgggaagggctactacattgagccaacaatattcactgatgtcacggatgagatgactattgcgaaggaagaaatatttgggcctgtgatgtcagtattcaaattcaagactgttgaggaggcaatcaagagagcaaatgcgaccaaatatggactggcagcgggcgtcatgactaacaacattaacatcgccaacaccgtcgcaagatcaatccgtgcgggtgctatctggataaattgttactttgccttcgacagagatagcccttacggaggctacaaaatgagtggtttcgggagagacatgggaatggatggcctcaagaagtatcttgcagttaaagctgttgctacccccatttataattcaccttggctgtaa

SEQ ID NO: 3 - DNA, 1341 bp, Gardenia jasminoides
atgaaggtactaatgttgccatggttagctcatggtcacatctctcctttcttagagctagccaagaggctggcaaagaaaaacttccacatctacctgtgttccacctctgtcaatctcagctccatcaagaacaagattaccggagaatattccgactcaatagaaccagttgagctacagcttccatgcttgcctgatcttcctcctcattaccacaccaccaatggcctcccaccccatctcatgaccaccctcaaaacagcctatgaactgtcagctcccgacttttctaatatcctcaccgctctgcatcctgacttggttgtgtacgactttaaccagccgtgggcagcagaaattgcttcgtctaaaaacatcccagcagttcaatttctcccggttggggcaacaatgatggctttcagtctgcacatgctcaagtattctggaaaagaattcccccacccagaaatttatatccgggactacgagatgctcaagtttcagtcaaggaacgatcaagttaatgatgttagtgatagagaaagaatcctgcaagctctggacctgtcgtgtaagattttgttggtcaagtcgttcaaagaaatcgaagaaaaattcatgaatactctctctgttgcatctggtaaaaaggtggtccccgttggccctcttgtccaagacgtcaatatcgatgacattcaagatgaggaaatggaaatcatccattggcttgaccaaaaggaaaatgcttcagtggtgtttgtctcttttggtagtgagtatttcttgactaaggaggaaagaaacgagattgctcggggtcttgagctcagcaatgttaactttatatgggtaattaggttccctctgggaggaaaaataactatggaagaagcattgcccgaaggttttcttgagagagtgggagatagaggaaaaattgtggatggatgggctcctcaggcaagaattttgaagcatgcgaatactggtgcttttttgagccattgtggatggagttcaatgatggagagtatgaaatttggtgttccaataatagctatgcctatgagtgttgatcaacctgtgaatgctagattgattgaagcagttggagtgggattggagcccttgagagacgagaaggggaatcttcaaagtgcggagattgccaaagtgattagaaaggttttggtggacgaaagtggagaaaatgtgaggaggaaggctaaggaattgagtgaacaaatggaaatgagaggtgacgaggaggagattgataaccttgtagaggagctgctgcaactctgccgaaagaacaacgggggctgttaa

SEQ ID NO: 4 - DNA, 1374 bp, Gardenia jasminoides
atgaattccagcaaagttcatgttttagttctgccatatcctgcccagggccacataaaccccttgctccagttctgtaaacgtttggtggcaaaaggtgtcaaaaccacgtttgtcaacactgtcttcgtctccaagtccattcaaccagatcccagctgctcaattaactttgagaccatttcagatggccatgacgaaggtggctatgcagcagctgaaagcccagaggcctatcttgtagaactggccaccttcggctcaaagacgttggctgatcttatcaggaagcttgaagacaagggcgaaccagtccaggccgtgatttatgattcattcctgacatgggctcttgatgtagctaagcaatttggacttgttacagctgcttttttcactcagacttgtgctgtaaacagcgtctactaccatgtttatcatggacttctaccgctccctctgtcagactcacctctttcacttcctggattgccgctgctccaacccaaggaaactccgtcctttgtttaccttcccgattcgtatcctgcttttcgtctcatgctcgttaatcagttctccaacgttgatcaagcagattgggtcatcctcaacattttccacaaattggaggaagatgtgctgaattggatagcgaaactttggcgagtgattacagtcggtccaacggttccatccatgtacttggataaacgccttgaggacgataaatgttacggaataaatctcttcaagccagactcctgcctgtgcatgaactggctaaataatcaaccaaaggactcggtagtttatgtatcattcggtagctggacagaaattgacgtaaaacaagtggaggaaatagcttcagctttgaaggaaagcggattcaaattcttgtgggtcgtgagatcatttgagaaggaaaagcttccaagcaacttcgctgaggagacgtcggagaaaggcttggtggtgacatggagtccacagcttgaggtattggcacatgaatccgtcgcttgtttcgtcactcattgcgggttcaattcagtgctggaggcgttgagtttaggggtgccggtggtggccgcgccgcagtggacggaccagcccaccaacgctaagtttctggaggatatttggggagttggtgtgaaggctggtgcggatgagaaaggaattgtgacgagggaaacgctagtttcctgcataagggagattatggagggagaaaaaggaaagcagattaaagagaatgccattaaatggaagactttagccaaagaagcagttgatgagggcggaagttctgataagaacattgacgaatttgttgcagaattggctggccagaaggcccagaactag

SEQ ID NO: 5 - protein, 664 aa, Gardenia jasminoides
MTDLLCFLYESLGAQHKYSPPLYTFTHPSIHLLLVLQNNNTKTAMDAFSSSFLSRLSQNPKLPTSLTNPSSPNIPLLHISSARIEDKPQPTIITSTPITATTPPSSNSNPLKKQNLPKYTLKRSNPKPQSSSQPPPSLQLQEPSRKPVEPSLLTKFFNALDNFIDTCIDPPTHPSVDPKYVLANNFVPVDELPPTECEVVEGFLPPCLDGAYFRNGPNPQFVTHGPYHFFDGDGMIHSIKISEGKATFCSRYVKTYKYMTERDTGSPVFPKVFSGFNGLTASAARVALAAARMLAGQFNRANGFGLANTSLALVGGKLFALGEPDLPYAVKLTQTGDLVTVGRHDFDGKLIASMTAHPKIDPETGEAFAFRYALMPPFLTFFRINPDGTKEPDVPIFSMTRPSFVHDLAITRKYAIFPDIQIGINPLQMIAGGPLVGSDPRKVPRLGVIPRYAADEAEMKWFDVPGLNLMHAVNAWDEDDGDGIVVVGTNSLPIEHVLRRMDLVHASMVKIKIDLKTGMVWKHPISTRSMEFGVINPAYVGKKNKYVYAAVVDPLPKVSGVVKLDLSASAGEHRDCVIASQLYEPECFGSEPFFVAKDPNNPNADEDDGYVVSYVHDENTGESRFLVMDAKSPSLEIVAAVKLPQRVPSGFHGLFVRESELNKL

SEQ ID NO: 6 - protein, 503 aa, Gardenia jasminoides
MAVQSNGNGSSDSHVKVPQIKFTKLFINGEFVDSVSGKTFETIDPRNGEVIAEIAEGGKEDVDLAVKAAREAFDHGPWPRLPGSERRKIMMKFADLIDENTQELATLDAIDAGKLFYLCKIMDIPGAAETIRYYAGAADKIHGETLKMSTALQGYTLHEPIGVVGHIIPWNFPSQMFAMKVGPALAAGCTMVVKPAEQTPLSALYYAHLAKLAGIPDGVLNVVTGFGQTAGAAISSHMDIDMVSFTGSTEVGRLVMQAAATSNLKPVCLELGGKSPILIFDDADVDKVTELALQGTLFNKGEICVAGSRIFVQEGIYDKFLIKLKQKVKNWVVGDPFDPTSHQGPQVDKKQYDRILSYIEHGKKEGATLFHGGKPCDGKGYYIEPTIFTDVTDEMTIAKEEIFGPVMSVFKFKTVEEAIKRANATKYGLAAGVMTNNINIANTVARSIRAGAIWINCYFAFDRDSPYGGYKMSGFGRDMGMDGLKKYLAVKAVATPIYNSPWL

SEQ ID NO: 7 - protein, 446 aa, Gardenia jasminoides
MKVLMLPWLAHGHISPFLELAKRLAKKNFHIYLCSTSVNLSSIKNKITGEYSDSIEPVELQLPCLPDLPPHYHTTNGLPPHLMTTLKTAYELSAPDFSNILTALHPDLVVYDFNQPWAAEIASSKNIPAVQFLPVGATMMAFSLHMLKYSGKEFPHPEIYIRDYEMLKFQSRNDQVNDVSDRERILQALDLSCKILLVKSFKEIEEKFMNTLSVASGKKVVPVGPLVQDVNIDDIQDEEMEIIHWLDQKENASVVFVSFGSEYFLTKEERNEIARGLELSNVNFIWVIRFPLGGKITMEEALPEGFLERVGDRGKIVDGWAPQARILKHANTGAFLSHCGWSSMMESMKFGVPIIAMPMSVDQPVNARLIEAVGVGLEPLRDEKGNLQSAEIAKVIRKVLVDESGENVRRKAKELSEQMEMRGDEEEIDNLVEELLQLCRKNNGGC

SEQ ID NO: 8 - protein, 457 aa, Gardenia jasminoides
MNSSKVHVLVLPYPAQGHINPLLQFCKRLVAKGVKTTFVNTVFVSKSIQPDPSCSINFETISDGHDEGGYAAAESPEAYLVELATFGSKTLADLIRKLEDKGEPVQAVIYDSFLTWALDVAKQFGLVTAAFFTQTCAVNSVYYHVYHGLLPLPLSDSPLSLPGLPLLQPKETPSFVYLPDSYPAFRLMLVNQFSNVDQADWVILNIFHKLEEDVLNWIAKLWRVITVGPTVPSMYLDKRLEDDKCYGINLFKPDSCLCMNWLNNQPKDSVVYVSFGSWTEIDVKQVEEIASALKESGFKFLWVVRSFEKEKLPSNFAEETSEKGLVVTWSPQLEVLAHESVACFVTHCGFNSVLEALSLGVPVVAAPQWTDQPTNAKFLEDIWGVGVKAGADEKGIVTRETLVSCIREIMEGEKGKQIKENAIKWKTLAKEAVDEGGSSDKNIDEFVAELAGQKAQN